European Patent Application EP 4 710 935 A2, published March 18, 2026. Title: Novel immunotherapeutic composition and uses thereof. Applicant: Monash University. Application WO PCT/AU2014/050249, filed September 25, 2014. The sequence listing filed with the application follows.

SEQUENCE LISTING (143 sequences)

SEQ ID NO: 1 - protein, 8 aa, synthetic construct
FQNLQNHR

SEQ ID NO: 2 - protein, 6 aa, synthetic construct
IVQIEA

SEQ ID NO: 3 - protein, 10 aa, synthetic construct
NEGVIVKVSK

SEQ ID NO: 4 - protein, 12 aa, synthetic construct
EVKPDKKNPQLQ

SEQ ID NO: 5 - protein, 6 aa, synthetic construct
EGALML

SEQ ID NO: 6 - protein, 7 aa, synthetic construct
IMPAAHP

SEQ ID NO: 7 - protein, 9 aa, synthetic construct
  SITE 4: note = MISC_FEATURE - X is cysteine or serine
LRPXEQHLM

SEQ ID NO: 8 - protein, 10 aa, synthetic construct
  SITE 6: note = MISC_FEATURE - X is cysteien or serine
  SITE 8: note = MISC_FEATURE - X is cysteien or serine
ENNQRXMXEA

SEQ ID NO: 9 - protein, 626 aa, synthetic construct
MRGRVSPLMLLLGILVLASVSATHAKSSPYQKKTENPCAQRCLQSCQQEPDDLKQKACESRCTKLEYDPRCVYDPRGHTGTTNQRSPPGERTRGRQPGDYDDDRRQPRREEGGRWGPAGPREREREEDWRQPREDWRRPSHQQPRKIRPEGREGEQEWGTPGSHVREETSRNNPFYFPSRRFSTRYGNQNGRIRVLQRFDQRSRQFQNLQNHRIVQIEAKPNTLVLPKHADADNILVIQQGQATVTVANGNNRKSFNLDEGHALRIPSGFISYILNRHDNQNLRVAKISMPVNTPGQFEDFFPASSRDQSSYLQGFSRNTLEAAFNAEFNEIRRVLLEENAGGEQEERGQRRWSTRSSENNEGVIVKVSKEHVEELTKHAKSVSKKGSEEEGDITNPINLREGEPDLSNNFGKLFEVKPDKKNPQLQDLDMMLTCVEIKEGALMLPHFNSKAMVIVVVNKGTGNLELVAVRKEQQQRGRREEEEDEDEEEEGSNREVRRYTARLKEGDVFIMPAAHPVAINASSELHLLGFGINAENNHRIFLAGDKDNVIDQIEKQAKDLAFPGSGEQVEKLIKNQKESHFVSARPQSQSQSPSSPEKESPEKEDQEEENQGGKGPLLSILKAFN

SEQ ID NO: 10 - protein, 157 aa, synthetic construct
LTILVALALFLLAAHASARQQWELQGDRRCQSQLERANLRPCEQHLMQKIQRDEDSYERDPYSPSQDPYSPSPYDRRGAGSSQHQERCCNELNEFENNQRCMCEALQQIMENQSDRLQGRQQEQQFKRELRNLPQQCGLRAPQRCDLDVESGGRDRY

SEQ ID NO: 11 - protein, 20 aa, synthetic construct
FQNLQNHRIVQIEAKPNTLV

SEQ ID NO: 12 - protein, 18 aa, synthetic construct
STRSSENNEGVIVKVSKE

SEQ ID NO: 13 - protein, 17 aa, synthetic construct
VEIKEGALMLPHFNSKA

SEQ ID NO: 14 - protein, 16 aa, synthetic construct
VFIMPAAHPVAINASS

SEQ ID NO: 15 - protein, 11 aa, synthetic construct
  SITE 6: note = MISC_FEATURE - X is cysteine or serine
ANLRPXEQHLM

SEQ ID NO: 16 - protein, 14 aa, synthetic construct
  SITE 8: note = MISC_FEATURE - X is cysteine or serine
  SITE 10: note = MISC_FEATURE - X is cysteine or serine
EFENNQRXMXEALQ

SEQ ID NO: 17 - protein, 19 aa, synthetic construct
NNFGKLFEVKPDKKNPQLQ

SEQ ID NO: 18 - protein, 19 aa, synthetic construct
GDVFIMPAAHPVAINASSE

SEQ ID NO: 19 - protein, 16 aa, synthetic construct
  SITE 11: note = MISC_FEATURE - X is cysteine or serine
SQLERANLRPXEQHLM

SEQ ID NO: 20 - protein, 17 aa, synthetic construct
  SITE 11: note = MISC_FEATURE - X is cysteine or serine
  SITE 13: note = MISC_FEATURE - X is cysteine or serine
ELNEFENNQRXMXEALQ

SEQ ID NO: 21 - protein, 10 aa, synthetic construct
FQNLQNHRIV

SEQ ID NO: 22 - protein, 13 aa, synthetic construct
RIVQIEAKPNTLV

SEQ ID NO: 23 - protein, 13 aa, synthetic construct
ENNEGVIVKVSKE

SEQ ID NO: 24 - protein, 13 aa, synthetic construct
EVKPDKKNPQLQD

SEQ ID NO: 25 - protein, 16 aa, synthetic construct
  SITE 8: note = MISC_FEATURE - X is cysteine or serine
  SITE 10: note = MISC_FEATURE - X is cysteine or serine
EFENNQRXMXEALQQI

SEQ ID NO: 26 - protein, 20 aa, synthetic construct
NNFGKLFEVKPDKKNPQLQD

SEQ ID NO: 27 - protein, 19 aa, synthetic construct
  SITE 11: note = MISC_FEATURE - X is cysteine or serine
  SITE 13: note = MISC_FEATURE - X is cysteine or serine
ELNEFENNQRXMXEALQQI

SEQ ID NO: 28 - protein, 19 aa, synthetic construct
WSTRSSENNEGVIVVKSKE

SEQ ID NO: 29 - protein, 18 aa, synthetic construct
GDVFIMPAAHPVAINASS

SEQ ID NO: 30 - protein, 18 aa, synthetic construct
STRSSENNEGVIVKVSKE

SEQ ID NO: 31 - protein, 11 aa, synthetic construct
ANLRPSEQHLM

SEQ ID NO: 32 - protein, 14 aa, synthetic construct
EFENNQRSMSEALQ

SEQ ID NO: 33 - protein, 16 aa, synthetic construct
EFENNQRSMSEALQQI

SEQ ID NO: 34 - protein, 17 aa, synthetic construct
ALMLPHFNSKAMVIVVV

SEQ ID NO: 35 - protein, 17 aa, synthetic construct
NNFGKLFEVKPDKKNPQ

SEQ ID NO: 36 - protein, 13 aa, synthetic construct
  SITE 11: note = MISC_FEATURE - X is cysteine or serine
SQLERANLRPXEQ

SEQ ID NO: 37 - protein, 12 aa, synthetic construct
  SITE 11: note = MISC_FEATURE - X is cysteine or serine
ELNEFENNQRXM

SEQ ID NO: 38 - protein, 20 aa, synthetic construct
NNFGKLFEVKPDKKNPQLQD

SEQ ID NO: 39 - protein, 19 aa, synthetic construct
ELNEFENNQRSMSEALQQI

SEQ ID NO: 40 - protein, 18 aa, synthetic construct
NNFGKLFEVKPDKKNPQL

SEQ ID NO: 41 - protein, 14 aa, synthetic construct
  SITE 11: note = MISC_FEATURE - X is cysteine or serine
SQLERANLRPXEQH

SEQ ID NO: 42 - protein, 21 aa, synthetic construct
KAMVIVVVNKGTGNLELVAVD

SEQ ID NO: 43 - protein, 14 aa, synthetic construct
  SITE 10: note = MISC_FEATURE - X is cysteine or serine
RELRNLPQQXGLRA

SEQ ID NO: 44 - protein, 11 aa, synthetic construct
KAMVIVVVNKG

SEQ ID NO: 45 - protein, 17 aa, synthetic construct
AMVIVVVNKGTGNLELV

SEQ ID NO: 46 - protein, 16 aa, synthetic construct
VVNKGTGNLELVAVRK

SEQ ID NO: 47 - protein, 20 aa, synthetic construct
FDQRSRQFQNLQNHRIVQIE

SEQ ID NO: 48 - protein, 20 aa, synthetic construct
NLQNHRIVQIEAKPNTLVLP

SEQ ID NO: 49 - protein, 20 aa, synthetic construct
RWSTRSSENNEGVIVKVSKE

SEQ ID NO: 50 - protein, 20 aa, synthetic construct
DLSNNFGKLFEVKPDKKNPQ

SEQ ID NO: 51 - protein, 20 aa, synthetic construct
FEVKPDKKNPQLQDLDMMLT

SEQ ID NO: 52 - protein, 20 aa, synthetic construct
LTCVEIKEGALMLPHFNSKA

SEQ ID NO: 53 - protein, 20 aa, synthetic construct
ALMLPHFNSKAMVIVVVNKG

SEQ ID NO: 54 - protein, 21 aa, synthetic construct
KAMVIVVVNKGTGNLELVAVA

SEQ ID NO: 55 - protein, 20 aa, synthetic construct
KEGDVFIMPAAHPVAINASS

SEQ ID NO: 56 - protein, 20 aa, synthetic construct
RRCQSQLERANLRPCEQHLM

SEQ ID NO: 57 - protein, 20 aa, synthetic construct
ANLRPCEQHLMQKIQRDEDS

SEQ ID NO: 58 - protein, 20 aa, synthetic construct
ELNEFENNQRCMCEALQQIM

SEQ ID NO: 59 - protein, 20 aa, synthetic construct
KRELRNLPQQCGLRAPQRCD

SEQ ID NO: 60 - protein, 8 aa, synthetic construct
FQNLQNHR

SEQ ID NO: 61 - protein, 10 aa, synthetic construct
FQNLQNHRIV

SEQ ID NO: 62 - protein, 10 aa, synthetic construct
RIVQIEAKPN

SEQ ID NO: 63 - protein, 13 aa, synthetic construct
RIVQIEAKPNTLV

SEQ ID NO: 64 - protein, 6 aa, synthetic construct
IVQIEA

SEQ ID NO: 65 - protein, 19 aa, synthetic construct
WSTRSSENNEGVIVKVSKE

SEQ ID NO: 66 - protein, 14 aa, synthetic construct
ENNEGVIVKVSKEA

SEQ ID NO: 67 - protein, 10 aa, synthetic construct
NEGVIVKVSK

SEQ ID NO: 68 - protein, 10 aa, synthetic construct
NNFGKLFEVK

SEQ ID NO: 69 - protein, 17 aa, synthetic construct
NNFGKLFEVKPDKKNPQ

SEQ ID NO: 70 - protein, 8 aa, synthetic construct
FGKLFEVK

SEQ ID NO: 71 - protein, 12 aa, synthetic construct
EVKPDKKNPQLQ

SEQ ID NO: 72 - protein, 10 aa, synthetic construct
VEIKEGALML

SEQ ID NO: 73 - protein, 14 aa, synthetic construct
VEIKEGALMLPHFN

SEQ ID NO: 74 - protein, 13 aa, synthetic construct
EGALMLPHFNSKA

SEQ ID NO: 75 - protein, 17 aa, synthetic construct
ALMLPHFNSKAMVIVVV

SEQ ID NO: 76 - protein, 15 aa, synthetic construct
LMLPHFNSKAMVIVV

SEQ ID NO: 77 - protein, 11 aa, synthetic construct
PHFNSKAMVIV

SEQ ID NO: 78 - protein, 9 aa, synthetic construct
KAMVIVVVN

SEQ ID NO: 79 - protein, 10 aa, synthetic construct
AMVIVVVNKG

SEQ ID NO: 80 - protein, 7 aa, synthetic construct
IVVVNKG

SEQ ID NO: 81 - protein, 16 aa, synthetic construct
AMVIVVVNKGTGNLEL

SEQ ID NO: 82 - protein, 17 aa, synthetic construct
AMVIVVVNKGTGNLELV

SEQ ID NO: 83 - protein, 13 aa, synthetic construct
VVNKGTGNLELVA

SEQ ID NO: 84 - protein, 14 aa, synthetic construct
VVNKGTGNLELVAV

SEQ ID NO: 85 - protein, 17 aa, synthetic construct
VEIKEGALMLPHFNSKA

SEQ ID NO: 86 - protein, 11 aa, synthetic construct
KAMVIVVVNKG

SEQ ID NO: 87 - protein, 19 aa, synthetic construct
AMVIVVVNKGTGNLELVAV

SEQ ID NO: 88 - protein, 18 aa, synthetic construct
GDVFIMPAAHPVAINASS

SEQ ID NO: 89 - protein, 16 aa, synthetic construct
VFIMPAAHPVAINASS

SEQ ID NO: 90 - protein, 12 aa, synthetic construct
FIMPAAHPVAIN

SEQ ID NO: 91 - protein, 7 aa, synthetic construct
IMPAAHP

SEQ ID NO: 92 - protein, 11 aa, synthetic construct
IMPAAHPVAIN

SEQ ID NO: 93 - protein, 20 aa, synthetic construct
RRCQSQLERANLRPCEQHLM

SEQ ID NO: 94 - protein, 13 aa, synthetic construct
SQLERANLRPCEQ

SEQ ID NO: 95 - protein, 11 aa, synthetic construct
SQLERANLRPC

SEQ ID NO: 96 - protein, 9 aa, synthetic construct
LERANLRPC

SEQ ID NO: 97 - protein, 11 aa, synthetic construct
LERANLRPCEQ

SEQ ID NO: 98 - protein, 10 aa, synthetic construct
ERANLRPCEQ

SEQ ID NO: 99 - protein, 11 aa, synthetic construct
ANLRPCEQHLM

SEQ ID NO: 100 - protein, 9 aa, synthetic construct
LRPCEQHLM

SEQ ID NO: 101 - protein, 20 aa, synthetic construct
ELNEFENNQRCMCEALQQIM

SEQ ID NO: 102 - protein, 12 aa, synthetic construct
ELNEFENNQRCM

SEQ ID NO: 103 - protein, 11 aa, synthetic construct
LNEFENNQRCM

SEQ ID NO: 104 - protein, 14 aa, synthetic construct
EFENNQRCMCEALQ

SEQ ID NO: 105 - protein, 10 aa, synthetic construct
ENNQRCMCEA

SEQ ID NO: 106 - protein, 11 aa, synthetic construct
NNQRCMCEALQ

SEQ ID NO: 107 - protein, 20 aa, synthetic construct
KRELRNLPQQCGLRAPQRCD

SEQ ID NO: 108 - protein, 12 aa, synthetic construct
RELRNLPQQCGL

SEQ ID NO: 109 - protein, 12 aa, synthetic construct
ELRNLPQQCGLR

SEQ ID NO: 110 - protein, 11 aa, synthetic construct
ELRNLPQQCGL

SEQ ID NO: 111 - protein, 10 aa, synthetic construct
LRNLPQQCGL

SEQ ID NO: 112 - protein, 9 aa, synthetic construct
LRNLPQQCG

SEQ ID NO: 113 - protein, 14 aa, synthetic construct
RELRNLPQQCGLRA

SEQ ID NO: 114 - protein, 20 aa, synthetic construct
FDQRSRQFQNLQNHRIVQIE

SEQ ID NO: 115 - protein, 20 aa, synthetic construct
NLQNHRIVQIEAKPNTLVLP

SEQ ID NO: 116 - protein, 20 aa, synthetic construct
DLSNNFGKLFEVKPDKKNPQ

SEQ ID NO: 117 - protein, 20 aa, synthetic construct
FEVKPDKKNPQLQDLDMMLT

SEQ ID NO: 118 - protein, 20 aa, synthetic construct
LTCVEIKEGALMLPHFNSKA

SEQ ID NO: 119 - protein, 20 aa, synthetic construct
ALMLPHFNSKAMVIVVVNKG

SEQ ID NO: 120 - protein, 20 aa, synthetic construct
KAMVIVVVNKGTGNLELVAV

SEQ ID NO: 121 - protein, 20 aa, synthetic construct
KEGDVFIMPAAHPVAINASS

SEQ ID NO: 122 - protein, 20 aa, synthetic construct
RRCQSQLERANLRPCEQHLM

SEQ ID NO: 123 - protein, 20 aa, synthetic construct
ELNEFENNQRCMCEALQQIM

SEQ ID NO: 124 - protein, 20 aa, synthetic construct
KRELRNLPQQCGLRAPQRCD

SEQ ID NO: 125 - protein, 9 aa, synthetic construct
LERANLRPC

SEQ ID NO: 126 - protein, 9 aa, synthetic construct
LRPCEQHLM

SEQ ID NO: 127 - protein, 9 aa, synthetic construct
FENNQRCMC

SEQ ID NO: 128 - protein, 10 aa, synthetic construct
LNEFENNQRC

SEQ ID NO: 129 - protein, 9 aa, synthetic construct
LRNLPQQCG

SEQ ID NO: 130 - protein, 9 aa, synthetic construct
LPQQCGLRA

SEQ ID NO: 131 - protein, 11 aa, synthetic construct
KAMVIVVVNKG

SEQ ID NO: 132 - protein, 16 aa, synthetic construct
VVNKGTGNLELVAVRK

SEQ ID NO: 133 - protein, 13 aa, synthetic construct
SQLERANLRPSEQ

SEQ ID NO: 134 - protein, 11 aa, synthetic construct
ANLRPSEQHLM

SEQ ID NO: 135 - protein, 12 aa, synthetic construct
ELNEFENNQRSM

SEQ ID NO: 136 - protein, 14 aa, synthetic construct
EFENNQRSMSEALQ

SEQ ID NO: 137 - protein, 9 aa, synthetic construct
LRPSEQHLM

SEQ ID NO: 138 - protein, 10 aa, synthetic construct
ENNQRSMSEA

SEQ ID NO: 139 - protein, 20 aa, synthetic construct
SQHQERCCNELNEFENNQRC

SEQ ID NO: 140 - protein, 14 aa, synthetic construct
EFENNQRCMCEALQ

SEQ ID NO: 141 - protein, 16 aa, synthetic construct
SQLERANLRPSEQHLM

SEQ ID NO: 142 - protein, 17 aa, synthetic construct
ELNEFENNQRSMSEALQ

SEQ ID NO: 143 - protein, 13 aa, synthetic construct
ENNEGVIVKVSKE